European Patent Application EP 4 257 603 A1, published October 11, 2023. Title: PHARMACEUTICAL COMPOSITION COMPRISING ANTI-CONNECTIVE TISSUE GROWTH FACTOR ANTIBODY. Applicant: Jiangsu Hengrui Pharmaceuticals Co., Ltd. Shanghai Hengrui Pharmaceutical Co., Ltd. The sequence listing filed with the application follows.

SEQUENCE LISTING (104 sequences)

SEQ ID NO: 1 - protein, 323 aa, Homo sapiens
  PEPTIDE: Full-length human CTGF protein
QNCSGPCRCPDEPAPRCPAGVSLVLDGCGCCRVCAKQLGELCTERDPCDPHKGLFCDFGSPANRKIGVCTAKDGAPCIFGGTVYRSGESFQSSCKYQCTCLDGAVGCMPLCSMDVRLPSPDCPFPRRVKLPGKCCEEWVCDEPKDQTVVGPALAAYRLEDTFGPDPTMIRANCLVQTTEWSACSKTCGMGISTRVTNDNASCRLEKQSRLCMVRPCEADLEENIKKGKKCIRTPKISKPIKFELSGCTSMKTYRAKFCGVCTDGRCCTPHRTTTLPVEFKCPDGEVMKKNMMFIKTCACHYNCPGDNDIFESLYYRKMYGDMA

SEQ ID NO: 2 - protein, 348 aa, Artificial Sequence
  PEPTIDE: CTGF-his
MEFGLSWLFLVAILKGVQCQNCSGPCRCPDEPAPRCPAGVSLVLDGCGCCRVCAKQLGELCTERDPCDPHKGLFCDFGSPANRKIGVCTAKDGAPCIFGGTVYRSGESFQSSCKYQCTCLDGAVGCMPLCSMDVRLPSPDCPFPRRVKLPGKCCEEWVCDEPKDQTVVGPALAAYRLEDTFGPDPTMIRANCLVQTTEWSACSKTCGMGISTRVTNDNASCRLEKQSRLCMVRPCEADLEENIKKGKKCIRTPKISKPIKFELSGCTSMKTYRAKFCGVCTDGRCCTPHRTTTLPVEFKCPDGEVMKKNMMFIKTCACHYNCPGDNDIFESLYYRKMYGDMAHHHHHH

SEQ ID NO: 3 - protein, 575 aa, Artificial Sequence
  PEPTIDE: mCTGF-Fc
MEFGLSWLFLVAILKGVQCQDCSAQCQCAAEAAPHCPAGVSLVLDGCGCCRVCAKQLGELCTERDPCDPHKGLFCDFGSPANRKIGVCTAKDGAPCVFGGSVYRSGESFQSSCKYQCTCLDGAVGCVPLCSMDVRLPSPDCPFPRRVKLPGKCCEEWVCDEPKDRTAVGPALAAYRLEDTFGPDPTMMRANCLVQTTEWSACSKTCGMGISTRVTNDNTFCRLEKQSRLCMVRPCEADLEENIKKGKKCIRTPKIAKPVKFELSGCTSVKTYRAKFCGVCTDGRCCTPHRTTTLPVEFKCPDGEIMKKNMMFIKTCACHYNCPGDNDIFESLYYRKMYGDMAEPRGPTIKPCPPCKCPAPNLLGGPSVFIFPPKIKDVLMISLSPIVTCVVVDVSEDDPDVQISWFVNNVEVHTAQTQTHREDYNSTLRVVSALPIQHQDWMSGKEFKCKVNNKDLPAPIERTISKPKGSVRAPQVYVLPPPEEEMTKKQVTLTCMVTDFMPEDIYVEWTNNGKTELNYKNTEPVLDSDGSYFMYSKLRVEKKNWVERNSYSCSVVHEGLHNHHTTKSFSRTPGK

SEQ ID NO: 4 - protein, 348 aa, Artificial Sequence
  PEPTIDE: Mouse CTGF protein-His tag
MEFGLSWLFLVAILKGVQCQDCSAQCQCAAEAAPHCPAGVSLVLDGCGCCRVCAKQLGELCTERDPCDPHKGLFCDFGSPANRKIGVCTAKDGAPCVFGGSVYRSGESFQSSCKYQCTCLDGAVGCVPLCSMDVRLPSPDCPFPRRVKLPGKCCEEWVCDEPKDRTAVGPALAAYRLEDTFGPDPTMMRANCLVQTTEWSACSKTCGMGISTRVTNDNTFCRLEKQSRLCMVRPCEADLEENIKKGKKCIRTPKIAKPVKFELSGCTSVKTYRAKFCGVCTDGRCCTPHRTTTLPVEFKCPDGEIMKKNMMFIKTCACHYNCPGDNDIFESLYYRKMYGDMAHHHHHH

SEQ ID NO: 5 - protein, 574 aa, Artificial Sequence
  PEPTIDE: Cynomolgus monkey CTGF-Fc
MEFGLSWLFLVAILKGVQCQNCSGPCRCPAEQAPRCPAGVSLVLDGCGCCRVCAKQLGELCTERDPCDPHKGLFCDFGSPANRKIGVCTAKDGAPCIFGGTVYRSGESFQSSCKYQCTCLDGAVGCMPLCSMDVRLPSPDCPFPRRVKLPGKCCEEWVCDEPKDQTVVGPALAAYRLEDTFGPDPTMIRANCLVQTTEWSACSKTCGMGISTRVTNDNASCRLEKQSRLCMVRPCEADLEENIKKGKKCIRTPKISKPIKFELSGCTSVKTYRAKFCGVCTDGRCCTPHRTTTLPVEFKCPDGEVMKKNMMFIKTCACHYNCPGDNDIFESLYYRKMYGDMAEPKSSDKTHTCPPCPAPELLGGPSVFLFPPKPKDTLMISRTPEVTCVVVDVSHEDPEVKFNWYVDGVEVHNAKTKPREEQYNSTYRVVSVLTVLHQDWLNGKEYKCKVSNKALPAPIEKTISKAKGQPREPQVYTLPPSRDELTKNQVSLTCLVKGFYPSDIAVEWESNGQPENNYKTTPPVLDSDGSFFLYSKLTVDKSRWQQGNVFSCSVMHEALHNHYTQKSLSLSPGK

SEQ ID NO: 6 - protein, 116 aa, Mus musculus
  DOMAIN: mab147 VH
EVQLVESGGGLVQPEGSLKLSCAASGFSFNTYAMNWVRQAPGKGLEWVARIRTKSNNYATYYADSVKDRFTISRDDSESMLYLQMNNLKTEDTAMYYCVETGFAYWDQGTLVTVSA

SEQ ID NO: 7 - protein, 106 aa, Mus musculus
  DOMAIN: mab147 VL
QIVLTQSPAIMSASPGEKVTITCSASSSVSYMHWFQQKPGTSPKLWIYSTSNLASGVPARFSGSGSGTSYSLTISRMEAEDAATYYCQQRSSYPLTFGAGTKLELK

SEQ ID NO: 8 - protein, 114 aa, Mus musculus
  DOMAIN: mab164 VH
QVQLKQSGPGLVQPSQSLSITCTVSGFSLTTFGVHWIRQSPGKGLEWLGVIWRRGGTDYNAAFMSRLSITKDNSRSHVFFKMTSLQTDDSAIYYCARDGGFDYWGQGTTLTVSS

SEQ ID NO: 9 - protein, 109 aa, Mus musculus
  DOMAIN: mab164 VL
QAVVTQESALTTSPGGTVILTCRSSIGAVTTSNYANWVQEKPDHLFTGLIGGTSNRAPGVPVRFSGSLIGDKAALTITGAQAEDDAMYFCALWYSTHYVFGGGTKVTVL

SEQ ID NO: 10 - protein, 5 aa, Mus musculus
  DOMAIN: mab147 HCDR1
TYAMN

SEQ ID NO: 11 - protein, 19 aa, Mus musculus
  DOMAIN: mab147 HCDR2
RIRTKSNNYATYYADSVKD

SEQ ID NO: 12 - protein, 5 aa, Mus musculus
  DOMAIN: mab147 HCDR3
TGFAY

SEQ ID NO: 13 - protein, 10 aa, Mus musculus
  DOMAIN: mab147 LCDR1
SASSSVSYMH

SEQ ID NO: 14 - protein, 7 aa, Mus musculus
  DOMAIN: mab147 LCDR2
STSNLAS

SEQ ID NO: 15 - protein, 9 aa, Mus musculus
  DOMAIN: mab147 LCDR3
QQRSSYPLT

SEQ ID NO: 16 - protein, 5 aa, Mus musculus
  DOMAIN: mab164 HCDR1
TFGVH

SEQ ID NO: 17 - protein, 16 aa, Mus musculus
  DOMAIN: mab164 HCDR2
VIWRRGGTDYNAAFMS

SEQ ID NO: 18 - protein, 6 aa, Mus musculus
  DOMAIN: mab164 HCDR3
DGGFDY

SEQ ID NO: 19 - protein, 14 aa, Mus musculus
  DOMAIN: mab164 LCDR1
RSSIGAVTTSNYAN

SEQ ID NO: 20 - protein, 7 aa, Mus musculus
  DOMAIN: mab164 LCDR2
GTSNRAP

SEQ ID NO: 21 - protein, 9 aa, Mus musculus
  DOMAIN: mab164 LCDR3
ALWYSTHYV

SEQ ID NO: 22 - protein, 106 aa, Artificial Sequence
  DOMAIN: Hu147-VL1
EIVLTQSPATLSLSPGERATLSCSASSSVSYMHWFQQKPGQSPRLLIYSTSNLASGIPARFSGSGSGTDYTLTISSLEPEDFAVYYCQQRSSYPLTFGQGTKLEIK

SEQ ID NO: 23 - protein, 106 aa, Artificial Sequence
  DOMAIN: Hu147-VL2
EIVLTQSPATLSLSPGERATLSCSASSSVSYMHWFQQKPGQSPKLLIYSTSNLASGIPARFSGSGSGTDYTLTISSLEPEDFAVYYCQQRSSYPLTFGQGTKLEIK

SEQ ID NO: 24 - protein, 106 aa, Artificial Sequence
  DOMAIN: Hu147-VL3
EIVLTQSPATLSLSPGERATLSCSASSSVSYMHWFQQKPGQSPKLWIYSTSNLASGVPARFSGSGSGTDYTLTISSLEPEDFAVYYCQQRSSYPLTFGQGTKLEIK

SEQ ID NO: 25 - protein, 106 aa, Artificial Sequence
  DOMAIN: Hu147-VL4
DIQMTQSPSSLSASVGDRVTITCSASSSVSYMHWFQQKPGKSPKLLIYSTSNLASGVPSRFSGSGSGTDYTLTISSLQPEDFATYYCQQRSSYPLTFGQGTKLEIK

SEQ ID NO: 26 - protein, 106 aa, Artificial Sequence
  DOMAIN: Hu147-VL5
DIQLTQSPSSLSASVGDRVTITCSASSSVSYMHWFQQKPGKSPKLWIYSTSNLASGVPSRFSGSGSGTDYTLTISSLQPEDFATYYCQQRSSYPLTFGQGTKLEIK

SEQ ID NO: 27 - protein, 116 aa, Artificial Sequence
  DOMAIN: Hu147-VH1
EVQLVESGGGLVQPGGSLRLSCAASGFTFSTYAMNWVRQAPGKGLEWVGRIRTKSNNYATYYADSVKDRFTISRDDSKNSLYLQMNSLKTEDTAVYYCVETGFAYWDQGTLVTVSS

SEQ ID NO: 28 - protein, 116 aa, Artificial Sequence
  DOMAIN: Hu147-VH2
EVQLVESGGGLVQPGGSLRLSCAASGFTFNTYAMNWVRQAPGKGLEWVARIRTKSNNYATYYADSVKDRFTISRDDSKNSLYLQMNSLKTEDTAVYYCVETGFAYWDQGTLVTVSS

SEQ ID NO: 29 - protein, 116 aa, Artificial Sequence
  DOMAIN: Hu147-VH3
EVQLVESGGGLVQPGGSLRLSCAASGFSFNTYAMNWVRQAPGKGLEWVARIRTKSNNYATYYADSVKDRFTISRDDSESSLYLQMNSLKTEDTAVYYCVETGFAYWDQGTLVTVSS

SEQ ID NO: 30 - protein, 109 aa, Artificial Sequence
  DOMAIN: Hu164-VL7
ETVVTQEPSLTVSPGGTVTLTCRSSIGAVTTSNYANWVQQKPGQAFRGLIGGTSNRAPWTPARFSGSLLGGKAALTLSGVQPEDEAEYYCALWYSTHYVFGGGTKLTVL

SEQ ID NO: 31 - protein, 109 aa, Artificial Sequence
  DOMAIN: Hu164-VL8
ETVVTQEPSFSVSPGGTVTLTCRSSIGAVTTSNYANWVQQTPGQAFRGLIGGTSNRAPGVPDRFSGSILGNKAALTITGAQADDESDYYCALWYSTHYVFGGGTKLTVL

SEQ ID NO: 32 - protein, 109 aa, Artificial Sequence
  DOMAIN: Hu164-VL9
ESVVTQPPSVSGAPGQRVTISCRSSIGAVTTSNYANWVQQLPGTAFKGLIGGTSNRAPGVPDRFSGSKSGTSASLAITGLQAEDEADYYCALWYSTHYVFGGGTKLTVL

SEQ ID NO: 33 - protein, 114 aa, Artificial Sequence
  DOMAIN: Hu164-VH5
EVTLKESGPVLVKPTETLTLTCTVSGFSLSTFGVHWIRQPPGKALEWLAVIWRRGGTDYNAAFMSRLTISKDTSKSQVVLTMTNMDPVDTATYYCARDGGFDYWGQGTTVTVSS

SEQ ID NO: 34 - protein, 114 aa, Artificial Sequence
  DOMAIN: Hu164-VH6
EVTLKESGPVLVKPTETLTLTCTVSGFSLSTFGVHWIRQPPGKGLEWLGVIWRRGGTDYNAAFMSRLTISKDTSKSQVVFTMTNMDPVDTATYYCARDGGFDYWGQGTTVTVSS

SEQ ID NO: 35 - protein, 114 aa, Artificial Sequence
  DOMAIN: Hu164-VH7
EVQLQESGPGLVKPSQTLSLTCTVSGFSISTFGVHWIRQHPGKGLEWIGVIWRRGGTDYNAAFMSRVTISKDTSKNQVSLKLSSVTAADTAVYYCARDGGFDYWGQGTTVTVSS

SEQ ID NO: 36 - protein, 114 aa, Artificial Sequence
  DOMAIN: Hu164-VH8
EVQLQESGPGLVKPSQTLSLTCTVSGFSISTFGVHWIRQHPGKGLEWLGVIWRRGGTDYNAAFMSRLTISKDTSKNQVSFKLSSVTAADTAVYYCARDGGFDYWGQGTTVTVSS

SEQ ID NO: 37 - protein, 330 aa, Artificial Sequence [sequence omitted]

SEQ ID NO: 38 - protein, 330 aa, Artificial Sequence
  DOMAIN: Heavy chain constant region y
ASTKGPSVFPLAPSSKSTSGGTAALGCLVKDYFPEPVTVSWNSGALTSGVHTFPAVLQSSGLYSLSSVVTVPSSSLGTQTYICNVNHKPSNTKVDKKVEPKSCDKTHTCPPCPAPELLGGPSVFLFPPKPKDTLYITREPEVTCVVVDVSHEDPEVKFNWYVDGVEVHNAKTKPREEQYNSTYRVVSVLTVLHQDWLNGKEYKCKVSNKALPAPIEKTISKAKGQPREPQVYTLPPSRDELTKNQVSLTCLVKGFYPSDIAVEWESNGQPENNYKTTPPVLDSDGSFFLYSKLTVDKSRWQQGNVFSCSVMHEALHNHYTQKSLSLSPGK

SEQ ID NO: 39 - protein, 107 aa, Artificial Sequence [sequence omitted]

SEQ ID NO: 40 - protein, 105 aa, Artificial Sequence
  DOMAIN: Humanized antibody light chain lambda constant region
GQPKANPTVTLFPPSSEELQANKATLVCLISDFYPGAVTVAWKADGSPVKAGVETTKPSKQSNNKYAASSYLSLTPEQWKSHRSYSCQVTHEGSTVEKTVAPTEC

SEQ ID NO: 41 - protein, 446 aa, Artificial Sequence
  CHAIN: Heavy chain of Ch147
EVQLVESGGGLVQPEGSLKLSCAASGFSFNTYAMNWVRQAPGKGLEWVARIRTKSNNYATYYADSVKDRFTISRDDSESMLYLQMNNLKTEDTAMYYCVETGFAYWDQGTLVTVSAASTKGPSVFPLAPSSKSTSGGTAALGCLVKDYFPEPVTVSWNSGALTSGVHTFPAVLQSSGLYSLSSVVTVPSSSLGTQTYICNVNHKPSNTKVDKKVEPKSCDKTHTCPPCPAPELLGGPSVFLFPPKPKDTLMISRTPEVTCVVVDVSHEDPEVKFNWYVDGVEVHNAKTKPREEQYNSTYRVVSVLTVLHQDWLNGKEYKCKVSNKALPAPIEKTISKAKGQPREPQVYTLPPSRDELTKNQVSLTCLVKGFYPSDIAVEWESNGQPENNYKTTPPVLDSDGSFFLYSKLTVDKSRWQQGNVFSCSVMHEALHNHYTQKSLSLSPGK

SEQ ID NO: 42 - protein, 213 aa, Artificial Sequence
  CHAIN: Light chain of Ch147
QIVLTQSPAIMSASPGEKVTITCSASSSVSYMHWFQQKPGTSPKLWIYSTSNLASGVPARFSGSGSGTSYSLTISRMEAEDAATYYCQQRSSYPLTFGAGTKLELKRTVAAPSVFIFPPSDEQLKSGTASVVCLLNNFYPREAKVQWKVDNALQSGNSQESVTEQDSKDSTYSLSSTLTLSKADYEKHKVYACEVTHQGLSSPVTKSFNRGEC

SEQ ID NO: 43 - protein, 446 aa, Artificial Sequence
  CHAIN: Heavy chain of Hu147-11wk
EVQLVESGGGLVQPGGSLRLSCAASGFTFSTYAMNWVRQAPGKGLEWVGRIRTKSNNYATYYADSVKDRFTISRDDSKNSLYLQMNSLKTEDTAVYYCVETGFAYWDQGTLVTVSSASTKGPSVFPLAPSSKSTSGGTAALGCLVKDYFPEPVTVSWNSGALTSGVHTFPAVLQSSGLYSLSSVVTVPSSSLGTQTYICNVNHKPSNTKVDKKVEPKSCDKTHTCPPCPAPELLGGPSVFLFPPKPKDTLMISRTPEVTCVVVDVSHEDPEVKFNWYVDGVEVHNAKTKPREEQYNSTYRVVSVLTVLHQDWLNGKEYKCKVSNKALPAPIEKTISKAKGQPREPQVYTLPPSRDELTKNQVSLTCLVKGFYPSDIAVEWESNGQPENNYKTTPPVLDSDGSFFLYSKLTVDKSRWQQGNVFSCSVMHEALHNHYTQKSLSLSPGK

SEQ ID NO: 44 - protein, 446 aa, Artificial Sequence
  CHAIN: Heavy chain of Hu147-21wk
EVQLVESGGGLVQPGGSLRLSCAASGFTFNTYAMNWVRQAPGKGLEWVARIRTKSNNYATYYADSVKDRFTISRDDSKNSLYLQMNSLKTEDTAVYYCVETGFAYWDQGTLVTVSSASTKGPSVFPLAPSSKSTSGGTAALGCLVKDYFPEPVTVSWNSGALTSGVHTFPAVLQSSGLYSLSSVVTVPSSSLGTQTYICNVNHKPSNTKVDKKVEPKSCDKTHTCPPCPAPELLGGPSVFLFPPKPKDTLMISRTPEVTCVVVDVSHEDPEVKFNWYVDGVEVHNAKTKPREEQYNSTYRVVSVLTVLHQDWLNGKEYKCKVSNKALPAPIEKTISKAKGQPREPQVYTLPPSRDELTKNQVSLTCLVKGFYPSDIAVEWESNGQPENNYKTTPPVLDSDGSFFLYSKLTVDKSRWQQGNVFSCSVMHEALHNHYTQKSLSLSPGK

SEQ ID NO: 45 - protein, 446 aa, Artificial Sequence
  CHAIN: Heavy chain of Hu147-31wk
EVQLVESGGGLVQPGGSLRLSCAASGFSFNTYAMNWVRQAPGKGLEWVARIRTKSNNYATYYADSVKDRFTISRDDSESSLYLQMNSLKTEDTAVYYCVETGFAYWDQGTLVTVSSASTKGPSVFPLAPSSKSTSGGTAALGCLVKDYFPEPVTVSWNSGALTSGVHTFPAVLQSSGLYSLSSVVTVPSSSLGTQTYICNVNHKPSNTKVDKKVEPKSCDKTHTCPPCPAPELLGGPSVFLFPPKPKDTLMISRTPEVTCVVVDVSHEDPEVKFNWYVDGVEVHNAKTKPREEQYNSTYRVVSVLTVLHQDWLNGKEYKCKVSNKALPAPIEKTISKAKGQPREPQVYTLPPSRDELTKNQVSLTCLVKGFYPSDIAVEWESNGQPENNYKTTPPVLDSDGSFFLYSKLTVDKSRWQQGNVFSCSVMHEALHNHYTQKSLSLSPGK

SEQ ID NO: 46 - protein, 446 aa, Artificial Sequence
  CHAIN: Heavy chain of Hu147-11yk
EVQLVESGGGLVQPGGSLRLSCAASGFTFSTYAMNWVRQAPGKGLEWVGRIRTKSNNYATYYADSVKDRFTISRDDSKNSLYLQMNSLKTEDTAVYYCVETGFAYWDQGTLVTVSSASTKGPSVFPLAPSSKSTSGGTAALGCLVKDYFPEPVTVSWNSGALTSGVHTFPAVLQSSGLYSLSSVVTVPSSSLGTQTYICNVNHKPSNTKVDKKVEPKSCDKTHTCPPCPAPELLGGPSVFLFPPKPKDTLYITREPEVTCVVVDVSHEDPEVKFNWYVDGVEVHNAKTKPREEQYNSTYRVVSVLTVLHQDWLNGKEYKCKVSNKALPAPIEKTISKAKGQPREPQVYTLPPSRDELTKNQVSLTCLVKGFYPSDIAVEWESNGQPENNYKTTPPVLDSDGSFFLYSKLTVDKSRWQQGNVFSCSVMHEALHNHYTQKSLSLSPGK

SEQ ID NO: 47 - protein, 446 aa, Artificial Sequence
  CHAIN: Heavy chain of Hu147-21yk
EVQLVESGGGLVQPGGSLRLSCAASGFTFNTYAMNWVRQAPGKGLEWVARIRTKSNNYATYYADSVKDRFTISRDDSKNSLYLQMNSLKTEDTAVYYCVETGFAYWDQGTLVTVSSASTKGPSVFPLAPSSKSTSGGTAALGCLVKDYFPEPVTVSWNSGALTSGVHTFPAVLQSSGLYSLSSVVTVPSSSLGTQTYICNVNHKPSNTKVDKKVEPKSCDKTHTCPPCPAPELLGGPSVFLFPPKPKDTLYITREPEVTCVVVDVSHEDPEVKFNWYVDGVEVHNAKTKPREEQYNSTYRVVSVLTVLHQDWLNGKEYKCKVSNKALPAPIEKTISKAKGQPREPQVYTLPPSRDELTKNQVSLTCLVKGFYPSDIAVEWESNGQPENNYKTTPPVLDSDGSFFLYSKLTVDKSRWQQGNVFSCSVMHEALHNHYTQKSLSLSPGK

SEQ ID NO: 48 - protein, 446 aa, Artificial Sequence
  CHAIN: Heavy chain of Hu147-31yk
EVQLVESGGGLVQPGGSLRLSCAASGFSFNTYAMNWVRQAPGKGLEWVARIRTKSNNYATYYADSVKDRFTISRDDSESSLYLQMNSLKTEDTAVYYCVETGFAYWDQGTLVTVSSASTKGPSVFPLAPSSKSTSGGTAALGCLVKDYFPEPVTVSWNSGALTSGVHTFPAVLQSSGLYSLSSVVTVPSSSLGTQTYICNVNHKPSNTKVDKKVEPKSCDKTHTCPPCPAPELLGGPSVFLFPPKPKDTLYITREPEVTCVVVDVSHEDPEVKFNWYVDGVEVHNAKTKPREEQYNSTYRVVSVLTVLHQDWLNGKEYKCKVSNKALPAPIEKTISKAKGQPREPQVYTLPPSRDELTKNQVSLTCLVKGFYPSDIAVEWESNGQPENNYKTTPPVLDSDGSFFLYSKLTVDKSRWQQGNVFSCSVMHEALHNHYTQKSLSLSPGK

SEQ ID NO: 49 - protein, 213 aa, Artificial Sequence
  CHAIN: Light chain of Hu147-11wk
EIVLTQSPATLSLSPGERATLSCSASSSVSYMHWFQQKPGQSPRLLIYSTSNLASGIPARFSGSGSGTDYTLTISSLEPEDFAVYYCQQRSSYPLTFGQGTKLEIKRTVAAPSVFIFPPSDEQLKSGTASVVCLLNNFYPREAKVQWKVDNALQSGNSQESVTEQDSKDSTYSLSSTLTLSKADYEKHKVYACEVTHQGLSSPVTKSFNRGEC

SEQ ID NO: 50 - protein, 213 aa, Artificial Sequence
  CHAIN: Light chain of Hu147-12wk
EIVLTQSPATLSLSPGERATLSCSASSSVSYMHWFQQKPGQSPKLLIYSTSNLASGIPARFSGSGSGTDYTLTISSLEPEDFAVYYCQQRSSYPLTFGQGTKLEIKRTVAAPSVFIFPPSDEQLKSGTASVVCLLNNFYPREAKVQWKVDNALQSGNSQESVTEQDSKDSTYSLSSTLTLSKADYEKHKVYACEVTHQGLSSPVTKSFNRGEC

SEQ ID NO: 51 - protein, 213 aa, Artificial Sequence
  CHAIN: Light chain of Hu147-13wk
EIVLTQSPATLSLSPGERATLSCSASSSVSYMHWFQQKPGQSPKLWIYSTSNLASGVPARFSGSGSGTDYTLTISSLEPEDFAVYYCQQRSSYPLTFGQGTKLEIKRTVAAPSVFIFPPSDEQLKSGTASVVCLLNNFYPREAKVQWKVDNALQSGNSQESVTEQDSKDSTYSLSSTLTLSKADYEKHKVYACEVTHQGLSSPVTKSFNRGEC

SEQ ID NO: 52 - protein, 213 aa, Artificial Sequence
  CHAIN: Light chain of Hu147-14wk
DIQMTQSPSSLSASVGDRVTITCSASSSVSYMHWFQQKPGKSPKLLIYSTSNLASGVPSRFSGSGSGTDYTLTISSLQPEDFATYYCQQRSSYPLTFGQGTKLEIKRTVAAPSVFIFPPSDEQLKSGTASVVCLLNNFYPREAKVQWKVDNALQSGNSQESVTEQDSKDSTYSLSSTLTLSKADYEKHKVYACEVTHQGLSSPVTKSFNRGEC

SEQ ID NO: 53 - protein, 213 aa, Artificial Sequence
  CHAIN: Light chain of Hu147-15wk
DIQLTQSPSSLSASVGDRVTITCSASSSVSYMHWFQQKPGKSPKLWIYSTSNLASGVPSRFSGSGSGTDYTLTISSLQPEDFATYYCQQRSSYPLTFGQGTKLEIKRTVAAPSVFIFPPSDEQLKSGTASVVCLLNNFYPREAKVQWKVDNALQSGNSQESVTEQDSKDSTYSLSSTLTLSKADYEKHKVYACEVTHQGLSSPVTKSFNRGEC

SEQ ID NO: 54 - protein, 444 aa, Artificial Sequence
  CHAIN: Heavy chain of Ch164
QVQLKQSGPGLVQPSQSLSITCTVSGFSLTTFGVHWIRQSPGKGLEWLGVIWRRGGTDYNAAFMSRLSITKDNSRSHVFFKMTSLQTDDSAIYYCARDGGFDYWGQGTTLTVSSASTKGPSVFPLAPSSKSTSGGTAALGCLVKDYFPEPVTVSWNSGALTSGVHTFPAVLQSSGLYSLSSVVTVPSSSLGTQTYICNVNHKPSNTKVDKKVEPKSCDKTHTCPPCPAPELLGGPSVFLFPPKPKDTLMISRTPEVTCVVVDVSHEDPEVKFNWYVDGVEVHNAKTKPREEQYNSTYRVVSVLTVLHQDWLNGKEYKCKVSNKALPAPIEKTISKAKGQPREPQVYTLPPSRDELTKNQVSLTCLVKGFYPSDIAVEWESNGQPENNYKTTPPVLDSDGSFFLYSKLTVDKSRWQQGNVFSCSVMHEALHNHYTQKSLSLSPGK

SEQ ID NO: 55 - protein, 214 aa, Artificial Sequence
  CHAIN: Light chain of Ch164
QAVVTQESALTTSPGGTVILTCRSSIGAVTTSNYANWVQEKPDHLFTGLIGGTSNRAPGVPVRFSGSLIGDKAALTITGAQAEDDAMYFCALWYSTHYVFGGGTKVTVLGQPKANPTVTLFPPSSEELQANKATLVCLISDFYPGAVTVAWKADGSPVKAGVETTKPSKQSNNKYAASSYLSLTPEQWKSHRSYSCQVTHEGSTVEKTVAPTEC

SEQ ID NO: 56 - protein, 444 aa, Artificial Sequence
  CHAIN: Heavy chain of Hu164-57wl
EVTLKESGPVLVKPTETLTLTCTVSGFSLSTFGVHWIRQPPGKALEWLAVIWRRGGTDYNAAFMSRLTISKDTSKSQVVLTMTNMDPVDTATYYCARDGGFDYWGQGTTVTVSSASTKGPSVFPLAPSSKSTSGGTAALGCLVKDYFPEPVTVSWNSGALTSGVHTFPAVLQSSGLYSLSSVVTVPSSSLGTQTYICNVNHKPSNTKVDKKVEPKSCDKTHTCPPCPAPELLGGPSVFLFPPKPKDTLMISRTPEVTCVVVDVSHEDPEVKFNWYVDGVEVHNAKTKPREEQYNSTYRVVSVLTVLHQDWLNGKEYKCKVSNKALPAPIEKTISKAKGQPREPQVYTLPPSRDELTKNQVSLTCLVKGFYPSDIAVEWESNGQPENNYKTTPPVLDSDGSFFLYSKLTVDKSRWQQGNVFSCSVMHEALHNHYTQKSLSLSPGK

SEQ ID NO: 57 - protein, 444 aa, Artificial Sequence
  CHAIN: Heavy chain of Hu164-67wl
EVTLKESGPVLVKPTETLTLTCTVSGFSLSTFGVHWIRQPPGKGLEWLGVIWRRGGTDYNAAFMSRLTISKDTSKSQVVFTMTNMDPVDTATYYCARDGGFDYWGQGTTVTVSSASTKGPSVFPLAPSSKSTSGGTAALGCLVKDYFPEPVTVSWNSGALTSGVHTFPAVLQSSGLYSLSSVVTVPSSSLGTQTYICNVNHKPSNTKVDKKVEPKSCDKTHTCPPCPAPELLGGPSVFLFPPKPKDTLMISRTPEVTCVVVDVSHEDPEVKFNWYVDGVEVHNAKTKPREEQYNSTYRVVSVLTVLHQDWLNGKEYKCKVSNKALPAPIEKTISKAKGQPREPQVYTLPPSRDELTKNQVSLTCLVKGFYPSDIAVEWESNGQPENNYKTTPPVLDSDGSFFLYSKLTVDKSRWQQGNVFSCSVMHEALHNHYTQKSLSLSPGK

SEQ ID NO: 58 - protein, 444 aa, Artificial Sequence
  CHAIN: Heavy chain of Hu164-77wl
EVQLQESGPGLVKPSQTLSLTCTVSGFSISTFGVHWIRQHPGKGLEWIGVIWRRGGTDYNAAFMSRVTISKDTSKNQVSLKLSSVTAADTAVYYCARDGGFDYWGQGTTVTVSSASTKGPSVFPLAPSSKSTSGGTAALGCLVKDYFPEPVTVSWNSGALTSGVHTFPAVLQSSGLYSLSSVVTVPSSSLGTQTYICNVNHKPSNTKVDKKVEPKSCDKTHTCPPCPAPELLGGPSVFLFPPKPKDTLMISRTPEVTCVVVDVSHEDPEVKFNWYVDGVEVHNAKTKPREEQYNSTYRVVSVLTVLHQDWLNGKEYKCKVSNKALPAPIEKTISKAKGQPREPQVYTLPPSRDELTKNQVSLTCLVKGFYPSDIAVEWESNGQPENNYKTTPPVLDSDGSFFLYSKLTVDKSRWQQGNVFSCSVMHEALHNHYTQKSLSLSPGK

SEQ ID NO: 59 - protein, 444 aa, Artificial Sequence
  CHAIN: Heavy chain of Hu164-87wl
EVQLQESGPGLVKPSQTLSLTCTVSGFSISTFGVHWIRQHPGKGLEWLGVIWRRGGTDYNAAFMSRLTISKDTSKNQVSFKLSSVTAADTAVYYCARDGGFDYWGQGTTVTVSSASTKGPSVFPLAPSSKSTSGGTAALGCLVKDYFPEPVTVSWNSGALTSGVHTFPAVLQSSGLYSLSSVVTVPSSSLGTQTYICNVNHKPSNTKVDKKVEPKSCDKTHTCPPCPAPELLGGPSVFLFPPKPKDTLMISRTPEVTCVVVDVSHEDPEVKFNWYVDGVEVHNAKTKPREEQYNSTYRVVSVLTVLHQDWLNGKEYKCKVSNKALPAPIEKTISKAKGQPREPQVYTLPPSRDELTKNQVSLTCLVKGFYPSDIAVEWESNGQPENNYKTTPPVLDSDGSFFLYSKLTVDKSRWQQGNVFSCSVMHEALHNHYTQKSLSLSPGK

SEQ ID NO: 60 - protein, 444 aa, Artificial Sequence
  CHAIN: Heavy chain of Hu164-57yl
EVTLKESGPVLVKPTETLTLTCTVSGFSLSTFGVHWIRQPPGKALEWLAVIWRRGGTDYNAAFMSRLTISKDTSKSQVVLTMTNMDPVDTATYYCARDGGFDYWGQGTTVTVSSASTKGPSVFPLAPSSKSTSGGTAALGCLVKDYFPEPVTVSWNSGALTSGVHTFPAVLQSSGLYSLSSVVTVPSSSLGTQTYICNVNHKPSNTKVDKKVEPKSCDKTHTCPPCPAPELLGGPSVFLFPPKPKDTLYITREPEVTCVVVDVSHEDPEVKFNWYVDGVEVHNAKTKPREEQYNSTYRVVSVLTVLHQDWLNGKEYKCKVSNKALPAPIEKTISKAKGQPREPQVYTLPPSRDELTKNQVSLTCLVKGFYPSDIAVEWESNGQPENNYKTTPPVLDSDGSFFLYSKLTVDKSRWQQGNVFSCSVMHEALHNHYTQKSLSLSPGK

SEQ ID NO: 61 - protein, 444 aa, Artificial Sequence
  CHAIN: Heavy chain of Hu164-67yl
EVTLKESGPVLVKPTETLTLTCTVSGFSLSTFGVHWIRQPPGKGLEWLGVIWRRGGTDYNAAFMSRLTISKDTSKSQVVFTMTNMDPVDTATYYCARDGGFDYWGQGTTVTVSSASTKGPSVFPLAPSSKSTSGGTAALGCLVKDYFPEPVTVSWNSGALTSGVHTFPAVLQSSGLYSLSSVVTVPSSSLGTQTYICNVNHKPSNTKVDKKVEPKSCDKTHTCPPCPAPELLGGPSVFLFPPKPKDTLYITREPEVTCVVVDVSHEDPEVKFNWYVDGVEVHNAKTKPREEQYNSTYRVVSVLTVLHQDWLNGKEYKCKVSNKALPAPIEKTISKAKGQPREPQVYTLPPSRDELTKNQVSLTCLVKGFYPSDIAVEWESNGQPENNYKTTPPVLDSDGSFFLYSKLTVDKSRWQQGNVFSCSVMHEALHNHYTQKSLSLSPGK

SEQ ID NO: 62 - protein, 444 aa, Artificial Sequence
  CHAIN: Heavy chain of Hu164-77yl
EVQLQESGPGLVKPSQTLSLTCTVSGFSISTFGVHWIRQHPGKGLEWIGVIWRRGGTDYNAAFMSRVTISKDTSKNQVSLKLSSVTAADTAVYYCARDGGFDYWGQGTTVTVSSASTKGPSVFPLAPSSKSTSGGTAALGCLVKDYFPEPVTVSWNSGALTSGVHTFPAVLQSSGLYSLSSVVTVPSSSLGTQTYICNVNHKPSNTKVDKKVEPKSCDKTHTCPPCPAPELLGGPSVFLFPPKPKDTLYITREPEVTCVVVDVSHEDPEVKFNWYVDGVEVHNAKTKPREEQYNSTYRVVSVLTVLHQDWLNGKEYKCKVSNKALPAPIEKTISKAKGQPREPQVYTLPPSRDELTKNQVSLTCLVKGFYPSDIAVEWESNGQPENNYKTTPPVLDSDGSFFLYSKLTVDKSRWQQGNVFSCSVMHEALHNHYTQKSLSLSPGK

SEQ ID NO: 63 - protein, 444 aa, Artificial Sequence
  CHAIN: Heavy chain of Hu164-87yl
EVQLQESGPGLVKPSQTLSLTCTVSGFSISTFGVHWIRQHPGKGLEWLGVIWRRGGTDYNAAFMSRLTISKDTSKNQVSFKLSSVTAADTAVYYCARDGGFDYWGQGTTVTVSSASTKGPSVFPLAPSSKSTSGGTAALGCLVKDYFPEPVTVSWNSGALTSGVHTFPAVLQSSGLYSLSSVVTVPSSSLGTQTYICNVNHKPSNTKVDKKVEPKSCDKTHTCPPCPAPELLGGPSVFLFPPKPKDTLYITREPEVTCVVVDVSHEDPEVKFNWYVDGVEVHNAKTKPREEQYNSTYRVVSVLTVLHQDWLNGKEYKCKVSNKALPAPIEKTISKAKGQPREPQVYTLPPSRDELTKNQVSLTCLVKGFYPSDIAVEWESNGQPENNYKTTPPVLDSDGSFFLYSKLTVDKSRWQQGNVFSCSVMHEALHNHYTQKSLSLSPGK

SEQ ID NO: 64 - protein, 214 aa, Artificial Sequence
  CHAIN: Light chain of Hu164-57wl
ETVVTQEPSLTVSPGGTVTLTCRSSIGAVTTSNYANWVQQKPGQAFRGLIGGTSNRAPWTPARFSGSLLGGKAALTLSGVQPEDEAEYYCALWYSTHYVFGGGTKLTVLGQPKANPTVTLFPPSSEELQANKATLVCLISDFYPGAVTVAWKADGSPVKAGVETTKPSKQSNNKYAASSYLSLTPEQWKSHRSYSCQVTHEGSTVEKTVAPTEC

SEQ ID NO: 65 - protein, 214 aa, Artificial Sequence
  CHAIN: Light chain of Hu164-58wl
ETVVTQEPSFSVSPGGTVTLTCRSSIGAVTTSNYANWVQQTPGQAFRGLIGGTSNRAPGVPDRFSGSILGNKAALTITGAQADDESDYYCALWYSTHYVFGGGTKLTVLGQPKANPTVTLFPPSSEELQANKATLVCLISDFYPGAVTVAWKADGSPVKAGVETTKPSKQSNNKYAASSYLSLTPEQWKSHRSYSCQVTHEGSTVEKTVAPTEC

SEQ ID NO: 66 - protein, 214 aa, Artificial Sequence
  CHAIN: Light chain of Hu164-59wl
ESVVTQPPSVSGAPGQRVTISCRSSIGAVTTSNYANWVQQLPGTAFKGLIGGTSNRAPGVPDRFSGSKSGTSASLAITGLQAEDEADYYCALWYSTHYVFGGGTKLTVLGQPKANPTVTLFPPSSEELQANKATLVCLISDFYPGAVTVAWKADGSPVKAGVETTKPSKQSNNKYAASSYLSLTPEQWKSHRSYSCQVTHEGSTVEKTVAPTEC

SEQ ID NO: 67 - protein, 450 aa, Artificial Sequence
  CHAIN: Heavy chain of mAb1
EGQLVQSGGGLVHPGGSLRLSCAGSGFTFSSYGMHWVRQAPGKGLEWVSGIGTGGGTYSTDSVKGRFTISRDNAKNSLYLQMNSLRAEDMAVYYCARGDYYGSGSFFDCWGQGTLVTVSSASTKGPSVFPLAPSSKSTSGGTAALGCLVKDYFPEPVTVSWNSGALTSGVHTFPAVLQSSGLYSLSSVVTVPSSSLGTQTYICNVNHKPSNTKVDKRVEPKSCDKTHTCPPCPAPELLGGPSVFLFPPKPKDTLMISRTPEVTCVVVDVSHEDPEVKFNWYVDGVEVHNAKTKPREEQYNSTYRVVSVLTVLHQDWLNGKEYKCKVSNKALPAPIEKTISKAKGQPREPQVYTLPPSREEMTKNQVSLTCLVKGFYPSDIAVEWESNGQPENNYKTTPPVLDSDGSFFLYSKLTVDKSRWQQGNVFSCSVMHEALHNHYTQKSLSLSPGK

SEQ ID NO: 68 - protein, 214 aa, Artificial Sequence
  CHAIN: Light chain of mAb1
DIQMTQSPSSLSASVGDRVTITCRASQGISSWLAWYQQKPEKAPKSLIYAASSLQSGVPSRFSGSGSGTDFTLTISSLQPEDFATYYCQQYNSYPPTFGQGTKLEIKRTVAAPSVFIFPPSDEQLKSGTASVVCLLNNFYPREAKVQWKVDNALQSGNSQESVTEQDSKDSTYSLSSTLTLSKADYEKHKVYACEVTHQGLSSPVTKSFNRGEC

SEQ ID NO: 69 - protein, 122 aa, Artificial Sequence
  CHAIN: mab95 VH
EVLLQQSGPVLVKPGPSVKISCKASGFTFTNYDIHWVKQSHGKSLEWIGLVYPYNGGTAYNQKFKDKATLTFDTSSSTAYMELNSLTSEDSAVYYCARWGLIPGTTSYFDVWGTGTTVTVSS

SEQ ID NO: 70 - protein, 106 aa, Artificial Sequence
  DOMAIN: mab95 VL
QIVLSQSPPILSASPGEKVTMTCRASSSVSYIHWYQQKPRSSPKPWIYATSNLASGVPARFSGSGSGTSYSLTISRVEAEDAATYYCQQWNSNPWTFGGGTRLEIK

SEQ ID NO: 71 - protein, 5 aa, Artificial Sequence
  DOMAIN: mab95 HCDR1
NYDIH

SEQ ID NO: 72 - protein, 17 aa, Artificial Sequence
  DOMAIN: mab95 HCDR2
LVYPYNGGTAYNQKFKD

SEQ ID NO: 73 - protein, 13 aa, Artificial Sequence
  DOMAIN: mab95 HCDR3
WGLIPGTTSYFDV

SEQ ID NO: 74 - protein, 10 aa, Artificial Sequence
  DOMAIN: mab95 LCDR1
RASSSVSYIH

SEQ ID NO: 75 - protein, 7 aa, Artificial Sequence
  DOMAIN: mab95 LCDR2
ATSNLAS

SEQ ID NO: 76 - protein, 9 aa, Artificial Sequence
  DOMAIN: mab95 LCDR3
QQWNSNPWT

SEQ ID NO: 77 - protein, 106 aa, Artificial Sequence
  CHAIN: Hu95-VL1
EIVLTQSPATLSLSPGERATLSCRASSSVSYIHWYQQKPGQAPRPWIYATSNLASGIPARFSGSGSGTDYTLTISRLEPEDFAVYYCQQWNSNPWTFGGGTKVEIK

SEQ ID NO: 78 - protein, 106 aa, Artificial Sequence
  CHAIN: Hu95-VL2
EIVLTQSPATLSLSPGERATLSCRASSSVSYIHWYQQKPGQSPRPWIYATSNLASGVPARFSGSGSGTSYTLTISRLEPEDFAVYYCQQWNSNPWTFGGGTKVEIK

SEQ ID NO: 79 - protein, 105 aa, Artificial Sequence
  CHAIN: Hu95-VL3
ESVLTQPPSVSGAPGQRVTISCRASSSVSYIHWYQQLPGTAPKPWIYATSNLASGVPDRFSGSKSGTSYSLAITGLQAEDEADYYCQQWNSNPWTFGGGTKVEIK

SEQ ID NO: 80 - protein, 105 aa, Artificial Sequence
  CHAIN: Hu95-VL4
EIVLTQPPSVSGAPGQRVTISCRASSSVSYIHWYQQLPGTSPKPWIYATSNLASGVPDRFSGSKSGTSYSLAITGLQAEDEADYYCQQWNSNPWTFGGGTKVEIK

SEQ ID NO: 81 - protein, 122 aa, Artificial Sequence
  CHAIN: Hu95-VH1
EVQLVQSGAEVKKPGASVKVSCKASGFTFTNYDIHWVRQAPGQRLEWMGLVYPYNGGTAYNQKFKDRVTLTFDTSASTAYMELSSLRSEDTAVYYCARWGLIPGTTSYFDVWGQGTTVTVSS

SEQ ID NO: 82 - protein, 122 aa, Artificial Sequence
  CHAIN: Hu95-VH2
EVQLVQSGAEVKKPGASVKVSCKASGFTFTNYDIHWVRQAPGQRLEWIGLVYPYNGGTAYNQKFKDRATLTFDTSASTAYMELSSLRSEDTAVYYCARWGLIPGTTSYFDVWGQGTTVTVSS

SEQ ID NO: 83 - protein, 122 aa, Artificial Sequence
  CHAIN: Hu95-VH3
EVQLVQSGAEVKKPGASVKVSCKASGFTFTNYDIHWVKQAPGQRLEWMGLVYPYNGGTAYNQKFKDKVTLTFDTSASTAYMELSSLRSEDTAVYYCARWGLIPGTTSYFDVWGQGTTVTVSS

SEQ ID NO: 84 - protein, 122 aa, Artificial Sequence
  CHAIN: Hu95-VH4
EVQLVQSGAEVKKPGASVKVSCKASGFTFTNYDIHWVKQAPGQRLEWIGLVYPYNGGTAYNQKFKDKATLTFDTSASTAYMELSSLRSEDTAVYYCARWGLIPGTTSYFDVWGQGTTVTVSS

SEQ ID NO: 85 - protein, 122 aa, Artificial Sequence
  CHAIN: Hu95-VH5
EVQLVQSGAEVKKPGASVKVSCRASGFTFTNYAIHWVKQAPGQRLEWMGLVYPYTGGTAYNQKFKDKVTLTFDTSASTAYMELSSLRSEDTAVYYCARWGMIPGTNSYFDVWGQGTTVTVSS

SEQ ID NO: 86 - protein, 452 aa, Artificial Sequence
  CHAIN: Heavy chain of Ch95
EVLLQQSGPVLVKPGPSVKISCKASGFTFTNYDIHWVKQSHGKSLEWIGLVYPYNGGTAYNQKFKDKATLTFDTSSSTAYMELNSLTSEDSAVYYCARWGLIPGTTSYFDVWGTGTTVTVSSASTKGPSVFPLAPSSKSTSGGTAALGCLVKDYFPEPVTVSWNSGALTSGVHTFPAVLQSSGLYSLSSVVTVPSSSLGTQTYICNVNHKPSNTKVDKKVEPKSCDKTHTCPPCPAPELLGGPSVFLFPPKPKDTLMISRTPEVTCVVVDVSHEDPEVKFNWYVDGVEVHNAKTKPREEQYNSTYRVVSVLTVLHQDWLNGKEYKCKVSNKALPAPIEKTISKAKGQPREPQVYTLPPSRDELTKNQVSLTCLVKGFYPSDIAVEWESNGQPENNYKTTPPVLDSDGSFFLYSKLTVDKSRWQQGNVFSCSVMHEALHNHYTQKSLSLSPGK

SEQ ID NO: 87 - protein, 213 aa, Artificial Sequence
  CHAIN: Light chain of Ch95
QIVLSQSPPILSASPGEKVTMTCRASSSVSYIHWYQQKPRSSPKPWIYATSNLASGVPARFSGSGSGTSYSLTISRVEAEDAATYYCQQWNSNPWTFGGGTRLEIKRTVAAPSVFIFPPSDEQLKSGTASVVCLLNNFYPREAKVQWKVDNALQSGNSQESVTEQDSKDSTYSLSSTLTLSKADYEKHKVYACEVTHQGLSSPVTKSFNRGEC

SEQ ID NO: 88 - protein, 452 aa, Artificial Sequence
  CHAIN: Heavy chain of Hu95-11wk
EVQLVQSGAEVKKPGASVKVSCKASGFTFTNYDIHWVRQAPGQRLEWMGLVYPYNGGTAYNQKFKDRVTLTFDTSASTAYMELSSLRSEDTAVYYCARWGLIPGTTSYFDVWGQGTTVTVSSASTKGPSVFPLAPSSKSTSGGTAALGCLVKDYFPEPVTVSWNSGALTSGVHTFPAVLQSSGLYSLSSVVTVPSSSLGTQTYICNVNHKPSNTKVDKKVEPKSCDKTHTCPPCPAPELLGGPSVFLFPPKPKDTLMISRTPEVTCVVVDVSHEDPEVKFNWYVDGVEVHNAKTKPREEQYNSTYRVVSVLTVLHQDWLNGKEYKCKVSNKALPAPIEKTISKAKGQPREPQVYTLPPSRDELTKNQVSLTCLVKGFYPSDIAVEWESNGQPENNYKTTPPVLDSDGSFFLYSKLTVDKSRWQQGNVFSCSVMHEALHNHYTQKSLSLSPGK

SEQ ID NO: 89 - protein, 452 aa, Artificial Sequence
  CHAIN: Heavy chain of Hu95-21wk
EVQLVQSGAEVKKPGASVKVSCKASGFTFTNYDIHWVRQAPGQRLEWIGLVYPYNGGTAYNQKFKDRATLTFDTSASTAYMELSSLRSEDTAVYYCARWGLIPGTTSYFDVWGQGTTVTVSSASTKGPSVFPLAPSSKSTSGGTAALGCLVKDYFPEPVTVSWNSGALTSGVHTFPAVLQSSGLYSLSSVVTVPSSSLGTQTYICNVNHKPSNTKVDKKVEPKSCDKTHTCPPCPAPELLGGPSVFLFPPKPKDTLMISRTPEVTCVVVDVSHEDPEVKFNWYVDGVEVHNAKTKPREEQYNSTYRVVSVLTVLHQDWLNGKEYKCKVSNKALPAPIEKTISKAKGQPREPQVYTLPPSRDELTKNQVSLTCLVKGFYPSDIAVEWESNGQPENNYKTTPPVLDSDGSFFLYSKLTVDKSRWQQGNVFSCSVMHEALHNHYTQKSLSLSPGK

SEQ ID NO: 90 - protein, 452 aa, Artificial Sequence
  CHAIN: Heavy chain of Hu95-31wk
EVQLVQSGAEVKKPGASVKVSCKASGFTFTNYDIHWVKQAPGQRLEWMGLVYPYNGGTAYNQKFKDKVTLTFDTSASTAYMELSSLRSEDTAVYYCARWGLIPGTTSYFDVWGQGTTVTVSSASTKGPSVFPLAPSSKSTSGGTAALGCLVKDYFPEPVTVSWNSGALTSGVHTFPAVLQSSGLYSLSSVVTVPSSSLGTQTYICNVNHKPSNTKVDKKVEPKSCDKTHTCPPCPAPELLGGPSVFLFPPKPKDTLMISRTPEVTCVVVDVSHEDPEVKFNWYVDGVEVHNAKTKPREEQYNSTYRVVSVLTVLHQDWLNGKEYKCKVSNKALPAPIEKTISKAKGQPREPQVYTLPPSRDELTKNQVSLTCLVKGFYPSDIAVEWESNGQPENNYKTTPPVLDSDGSFFLYSKLTVDKSRWQQGNVFSCSVMHEALHNHYTQKSLSLSPGK

SEQ ID NO: 91 - protein, 452 aa, Artificial Sequence
  CHAIN: Heavy chain of Hu95-41wk
EVQLVQSGAEVKKPGASVKVSCKASGFTFTNYDIHWVKQAPGQRLEWIGLVYPYNGGTAYNQKFKDKATLTFDTSASTAYMELSSLRSEDTAVYYCARWGLIPGTTSYFDVWGQGTTVTVSSASTKGPSVFPLAPSSKSTSGGTAALGCLVKDYFPEPVTVSWNSGALTSGVHTFPAVLQSSGLYSLSSVVTVPSSSLGTQTYICNVNHKPSNTKVDKKVEPKSCDKTHTCPPCPAPELLGGPSVFLFPPKPKDTLMISRTPEVTCVVVDVSHEDPEVKFNWYVDGVEVHNAKTKPREEQYNSTYRVVSVLTVLHQDWLNGKEYKCKVSNKALPAPIEKTISKAKGQPREPQVYTLPPSRDELTKNQVSLTCLVKGFYPSDIAVEWESNGQPENNYKTTPPVLDSDGSFFLYSKLTVDKSRWQQGNVFSCSVMHEALHNHYTQKSLSLSPGK

SEQ ID NO: 92 - protein, 452 aa, Artificial Sequence
  CHAIN: Heavy chain of Hu95-51wk
EVQLVQSGAEVKKPGASVKVSCRASGFTFTNYAIHWVKQAPGQRLEWMGLVYPYTGGTAYNQKFKDKVTLTFDTSASTAYMELSSLRSEDTAVYYCARWGMIPGTNSYFDVWGQGTTVTVSSASTKGPSVFPLAPSSKSTSGGTAALGCLVKDYFPEPVTVSWNSGALTSGVHTFPAVLQSSGLYSLSSVVTVPSSSLGTQTYICNVNHKPSNTKVDKKVEPKSCDKTHTCPPCPAPELLGGPSVFLFPPKPKDTLMISRTPEVTCVVVDVSHEDPEVKFNWYVDGVEVHNAKTKPREEQYNSTYRVVSVLTVLHQDWLNGKEYKCKVSNKALPAPIEKTISKAKGQPREPQVYTLPPSRDELTKNQVSLTCLVKGFYPSDIAVEWESNGQPENNYKTTPPVLDSDGSFFLYSKLTVDKSRWQQGNVFSCSVMHEALHNHYTQKSLSLSPGK

SEQ ID NO: 93 - protein, 452 aa, Artificial Sequence
  CHAIN: Heavy chain of Hu95-11yk
EVQLVQSGAEVKKPGASVKVSCKASGFTFTNYDIHWVRQAPGQRLEWMGLVYPYNGGTAYNQKFKDRVTLTFDTSASTAYMELSSLRSEDTAVYYCARWGLIPGTTSYFDVWGQGTTVTVSSASTKGPSVFPLAPSSKSTSGGTAALGCLVKDYFPEPVTVSWNSGALTSGVHTFPAVLQSSGLYSLSSVVTVPSSSLGTQTYICNVNHKPSNTKVDKKVEPKSCDKTHTCPPCPAPELLGGPSVFLFPPKPKDTLYITREPEVTCVVVDVSHEDPEVKFNWYVDGVEVHNAKTKPREEQYNSTYRVVSVLTVLHQDWLNGKEYKCKVSNKALPAPIEKTISKAKGQPREPQVYTLPPSRDELTKNQVSLTCLVKGFYPSDIAVEWESNGQPENNYKTTPPVLDSDGSFFLYSKLTVDKSRWQQGNVFSCSVMHEALHNHYTQKSLSLSPGK

SEQ ID NO: 94 - protein, 452 aa, Artificial Sequence
  CHAIN: Heavy chain of Hu95-21yk
EVQLVQSGAEVKKPGASVKVSCKASGFTFTNYDIHWVRQAPGQRLEWIGLVYPYNGGTAYNQKFKDRATLTFDTSASTAYMELSSLRSEDTAVYYCARWGLIPGTTSYFDVWGQGTTVTVSSASTKGPSVFPLAPSSKSTSGGTAALGCLVKDYFPEPVTVSWNSGALTSGVHTFPAVLQSSGLYSLSSVVTVPSSSLGTQTYICNVNHKPSNTKVDKKVEPKSCDKTHTCPPCPAPELLGGPSVFLFPPKPKDTLYITREPEVTCVVVDVSHEDPEVKFNWYVDGVEVHNAKTKPREEQYNSTYRVVSVLTVLHQDWLNGKEYKCKVSNKALPAPIEKTISKAKGQPREPQVYTLPPSRDELTKNQVSLTCLVKGFYPSDIAVEWESNGQPENNYKTTPPVLDSDGSFFLYSKLTVDKSRWQQGNVFSCSVMHEALHNHYTQKSLSLSPGK

SEQ ID NO: 95 - protein, 452 aa, Artificial Sequence
  CHAIN: Hu95-31yk
EVQLVQSGAEVKKPGASVKVSCKASGFTFTNYDIHWVKQAPGQRLEWMGLVYPYNGGTAYNQKFKDKVTLTFDTSASTAYMELSSLRSEDTAVYYCARWGLIPGTTSYFDVWGQGTTVTVSSASTKGPSVFPLAPSSKSTSGGTAALGCLVKDYFPEPVTVSWNSGALTSGVHTFPAVLQSSGLYSLSSVVTVPSSSLGTQTYICNVNHKPSNTKVDKKVEPKSCDKTHTCPPCPAPELLGGPSVFLFPPKPKDTLYITREPEVTCVVVDVSHEDPEVKFNWYVDGVEVHNAKTKPREEQYNSTYRVVSVLTVLHQDWLNGKEYKCKVSNKALPAPIEKTISKAKGQPREPQVYTLPPSRDELTKNQVSLTCLVKGFYPSDIAVEWESNGQPENNYKTTPPVLDSDGSFFLYSKLTVDKSRWQQGNVFSCSVMHEALHNHYTQKSLSLSPGK

SEQ ID NO: 96 - protein, 452 aa, Artificial Sequence
  CHAIN: Heavy chain of Hu95-41yk
EVQLVQSGAEVKKPGASVKVSCKASGFTFTNYDIHWVKQAPGQRLEWIGLVYPYNGGTAYNQKFKDKATLTFDTSASTAYMELSSLRSEDTAVYYCARWGLIPGTTSYFDVWGQGTTVTVSSASTKGPSVFPLAPSSKSTSGGTAALGCLVKDYFPEPVTVSWNSGALTSGVHTFPAVLQSSGLYSLSSVVTVPSSSLGTQTYICNVNHKPSNTKVDKKVEPKSCDKTHTCPPCPAPELLGGPSVFLFPPKPKDTLYITREPEVTCVVVDVSHEDPEVKFNWYVDGVEVHNAKTKPREEQYNSTYRVVSVLTVLHQDWLNGKEYKCKVSNKALPAPIEKTISKAKGQPREPQVYTLPPSRDELTKNQVSLTCLVKGFYPSDIAVEWESNGQPENNYKTTPPVLDSDGSFFLYSKLTVDKSRWQQGNVFSCSVMHEALHNHYTQKSLSLSPGK

SEQ ID NO: 97 - protein, 452 aa, Artificial Sequence
  CHAIN: Heavy chain of Hu95-51yk
EVQLVQSGAEVKKPGASVKVSCRASGFTFTNYAIHWVKQAPGQRLEWMGLVYPYTGGTAYNQKFKDKVTLTFDTSASTAYMELSSLRSEDTAVYYCARWGMIPGTNSYFDVWGQGTTVTVSSASTKGPSVFPLAPSSKSTSGGTAALGCLVKDYFPEPVTVSWNSGALTSGVHTFPAVLQSSGLYSLSSVVTVPSSSLGTQTYICNVNHKPSNTKVDKKVEPKSCDKTHTCPPCPAPELLGGPSVFLFPPKPKDTLYITREPEVTCVVVDVSHEDPEVKFNWYVDGVEVHNAKTKPREEQYNSTYRVVSVLTVLHQDWLNGKEYKCKVSNKALPAPIEKTISKAKGQPREPQVYTLPPSRDELTKNQVSLTCLVKGFYPSDIAVEWESNGQPENNYKTTPPVLDSDGSFFLYSKLTVDKSRWQQGNVFSCSVMHEALHNHYTQKSLSLSPGK

SEQ ID NO: 98 - protein, 213 aa, Artificial Sequence
  CHAIN: Light chain of Hu95-11wk
EIVLTQSPATLSLSPGERATLSCRASSSVSYIHWYQQKPGQAPRPWIYATSNLASGIPARFSGSGSGTDYTLTISRLEPEDFAVYYCQQWNSNPWTFGGGTKVEIKRTVAAPSVFIFPPSDEQLKSGTASVVCLLNNFYPREAKVQWKVDNALQSGNSQESVTEQDSKDSTYSLSSTLTLSKADYEKHKVYACEVTHQGLSSPVTKSFNRGEC

SEQ ID NO: 99 - protein, 213 aa, Artificial Sequence
  CHAIN: Light chain of Hu95-12wk
EIVLTQSPATLSLSPGERATLSCRASSSVSYIHWYQQKPGQSPRPWIYATSNLASGVPARFSGSGSGTSYTLTISRLEPEDFAVYYCQQWNSNPWTFGGGTKVEIKRTVAAPSVFIFPPSDEQLKSGTASVVCLLNNFYPREAKVQWKVDNALQSGNSQESVTEQDSKDSTYSLSSTLTLSKADYEKHKVYACEVTHQGLSSPVTKSFNRGEC

SEQ ID NO: 100 - protein, 212 aa, Artificial Sequence
  CHAIN: Light chain of Hu95-13wk
ESVLTQPPSVSGAPGQRVTISCRASSSVSYIHWYQQLPGTAPKPWIYATSNLASGVPDRFSGSKSGTSYSLAITGLQAEDEADYYCQQWNSNPWTFGGGTKVEIKRTVAAPSVFIFPPSDEQLKSGTASVVCLLNNFYPREAKVQWKVDNALQSGNSQESVTEQDSKDSTYSLSSTLTLSKADYEKHKVYACEVTHQGLSSPVTKSFNRGEC

SEQ ID NO: 101 - protein, 212 aa, Artificial Sequence
  CHAIN: Light chain of Hu95-14wk
EIVLTQPPSVSGAPGQRVTISCRASSSVSYIHWYQQLPGTSPKPWIYATSNLASGVPDRFSGSKSGTSYSLAITGLQAEDEADYYCQQWNSNPWTFGGGTKVEIKRTVAAPSVFIFPPSDEQLKSGTASVVCLLNNFYPREAKVQWKVDNALQSGNSQESVTEQDSKDSTYSLSSTLTLSKADYEKHKVYACEVTHQGLSSPVTKSFNRGEC

SEQ ID NO: 102 - protein, 5 aa, Artificial Sequence
  DOMAIN: Hu95-VH5 HCDR1
NYAIH

SEQ ID NO: 103 - protein, 17 aa, Artificial Sequence
  DOMAIN: Hu95-VH5 HCDR2
LVYPYTGGTAYNQKFKD

SEQ ID NO: 104 - protein, 13 aa, Artificial Sequence
  DOMAIN: Hu95-VH5 HCDR3
WGMIPGTNSYFDV